European Patent Specification EP 3 574 099 B1, published October 25, 2023. Title: PROMOTER CONSTRUCT FOR CELL-FREE PROTEIN SYNTHESIS. Applicant: Fraunhofer -Gesellschaft zur Förderung der angewandten Forschung e.V. The sequence listing filed with the application follows.

SEQUENCE LISTING (15 sequences)

SEQ ID NO: 1 - DNA, 91 bp, Artificial Sequence
  promoter construct without an enhancing element between the T7 promoter element and the 5'UTR sequence element
taatacgactcactatagtatttttacaacaattaccaacaacaacaacaaacaacaacaacattacattttacattctacaactaccatg

SEQ ID NO: 2 - DNA, 94 bp, Artificial Sequence
  promoter construct having only three nucleic acids between the T7 promoter element and the 5'UTR sequence element
taatacgactcactatagaagtatttttacaacaattaccaacaacaacaacaaacaacaacaacattacattttacattctacaactaccatg

SEQ ID NO: 3 - DNA, 97 bp, Artificial Sequence
  DNA promoter construct according to the present disclosure
taatacgactcactatagggagagtatttttacaacaattaccaacaacaacaacaaacaacaacaacattacattttacattctacaactaccatg

SEQ ID NO: 4 - DNA, 97 bp, Artificial Sequence
  DNA promoter construct according to the present disclosure
taatacgactcactatagcaagagtatttttacaacaattaccaacaacaacaacaaacaacaacaacattacattttacattctacaactaccatg

SEQ ID NO: 5 - DNA, 97 bp, Artificial Sequence
  Promoter construct prior art
taatacgactcactatagaaagagtatttttacaacaattaccaacaacaacaacaaacaacaacaacattacattttacattctacaactaccatg

SEQ ID NO: 6 - DNA, 17 bp, Artificial Sequence
  Promoter sequence of T7 RNA polymerase without the original transcription start site
taatacgactcactata

SEQ ID NO: 7 - DNA, 17 bp, Artificial Sequence
  Promoter sequence of T3 RNA polymerase without the original transcription start site
aattaaccctcactaaa

SEQ ID NO: 8 - DNA, 18 bp, Artificial Sequence
  Promoter sequence of SP6 RNA polymerase without the original transcription start site
aatttaggtgacactata

SEQ ID NO: 9 - DNA, 17 bp, Artificial Sequence
  Promotor sequence of K11 RNA polymerase without the original transcription start site
aattagggcacactata

SEQ ID NO: 10 - DNA, 17 bp, Artificial Sequence
  Promoter sequence of BA14 RNA polymerase without the original transcription start site
taatacgactcactaat

SEQ ID NO: 11 - DNA, 20 bp, Artificial Sequence
  Promoter sequence of T7 RNA polymerase
taatacgactcactataggg

SEQ ID NO: 12 - DNA, 20 bp, Artificial Sequence
  Promoter sequence of T3 RNA polymerase
aattaaccctcactaaaggg

SEQ ID NO: 13 - DNA, 21 bp, Artificial Sequence
  Promoter sequence of SP6 RNA polymerase
aatttaggtgacactatagaa

SEQ ID NO: 14 - DNA, 71 bp, Tobacco mosaic virus
gtatttttacaacaattaccaacaacaacaacaaacaacaacaacattacattttacattctacaactaca

SEQ ID NO: 15 - DNA, 143 bp, Tobacco etch virus
aaataacaaatctcaacacaacatatacaaaacaaacgaatctcaagcaatcaagcattctacttctattgcagcaatttaaatcatttcttttaaagcaaaagcaattttctgaaaattttcaccatttacgaacgatagca